European Patent Specification EP 4 092 043 B1, published June 18, 2025. Title: Novel sugar porter family MFS transporter variant and a method for producing L-valine using the same. Applicant: CJ CheilJedang Corporation. The sequence listing filed with the application follows.

SEQUENCE LISTING (10 sequences)

SEQ ID NO: 1 - protein, 491 aa, Artificial Sequence
  sugar porter family MFS transporter, iolT1 variant
MASTFIQADSPEKSKKLPPLTEGPYRKRLFYVALVATFGGLLFGYDTGVINGALNPMTRELGLTAFTEGVVTSSLLFGAAAGAMFFGRISDNWGRRKTIISLAVAFFIGTMICVFAPSFAVMVVGRVLLGLAVGGASTVVPVYLAELAPFEIRGSLAGRNELMIVVGQLAAFVINAIIGNVFGHHDGVWRYMLAIAAIPAIALFFGMLRVPESPRWLVERGRIDEARAVLETIRPLERAHAEVADVEHLAKEEHVISEKSMGLREILSSKWLVRILLVGIGLGVAQQLTGINSIMYYGQVVLIEAGFSENAALIVNVAPGVIAVVGAFIALWMMDRINRRTTLITGYSLTTISHVLIGIASVAFPVGDPLRPYVILTLVVVFVGSMQTFLNVATWVMLSELFPLAMRGFAIGISVFFLWIANAFLGLFFPTIMEAVGLTGTFFMFAGIGVVALIFIYTQVPETRGRTLEEIDADVTSGVIFNKDIRKGKVH

SEQ ID NO: 2 - DNA, 1476 bp, Artificial Sequence
  sugar porter family MFS transporter, iolT1 variant coding gene
atggctagtaccttcattcaggccgacagccctgaaaaaagtaagaagctgcccccactcacagaaggtccgtatagaaaacggctattctacgttgcactagttgcgacgttcggtggactgctcttcggatacgacaccggcgtaatcaacggtgcactcaacccaatgacacgtgagctcgggctaaccgcgttcactgagggtgttgtaacttcttctctgctgtttggtgcagcagctggtgcgatgtttttcggtcgtatttccgacaactggggtcgtcggaaaacaatcatctcacttgcagtagctttctttatcggcaccatgatctgcgtgtttgctccatcttttgcagtaatggttgtcggacgtgtgcttcttggactcgcagttggtggcgcttccactgttgtccctgtctacctggctgaacttgctccttttgaaatccgtggctcactggctggccgtaatgagttgatgattgttgttggtcagctcgcagcttttgtcatcaatgcgattattggaaatgtttttggacaccacgatggtgtgtggcgctacatgctggcaattgccgcaatcccagcaattgccctcttctttggaatgctccgagttccagaatccccacgctggcttgttgagcgaggacgcattgatgaggctcgcgcagttcttgaaaccattcgccctcttgaacgtgcccatgcagaagttgctgatgttgaacacctagcaaaagaagaacatgtcatttccgagaagtccatgggcttaagggaaattttgtccagcaagtggcttgtgcgcatcctcctggtaggtatcggattgggtgtcgcacagcagctgaccggcattaactccatcatgtattacggccaggttgttctcattgaggctggtttctccgaaaatgcagctctgatcgtcaacgtggcacctggagttatcgcagttgtcggtgcattcatcgcactgtggatgatggatcgcatcaaccgccgtaccaccctcattaccggctactctctcaccaccattagccacgtgttgatcggcatcgcatccgtagcattcccagttggcgatccacttcgcccatacgttatcttgactctagttgtggtcttcgtaggatccatgcagaccttcctcaacgtagccacctgggtcatgctctccgagctcttcccgctggcaatgcgcggtttcgcaatcggtatctcagtgttcttcctttggatcgcaaacgcgttcctcggattgttcttcccaaccatcatggaagcagtaggactaaccggaaccttcttcatgttcgccggaatcggtgtggttgccttgatcttcatctacacccaggttccagaaacccgtggacgcaccttggaggagatcgatgcggatgttacttccggagtcatcttcaacaaggatatccggaagggaaaggtgcactaa

SEQ ID NO: 3 - protein, 491 aa, Artificial Sequence
  Wild-type sugar porter family MFS transporter, iolT1
MASTFIQADSPEKSKKLPPLTEGPYRKRLFYVALVATFGGLLFGYDTGVINGALNPMTRELGLTAFTEGVVTSSLLFGAAAGAMFFGRISDNWGRRKTIISLAVAFFIGTMICVFAPSFAVMVVGRVLLGLAVGGASTVVPVYLAELAPFEIRGSLAGRNELMIVVGQLAAFVINAIIGNVFGHHDGVWRYMLAIAAIPAIALFFGMLRVPESPRWLVERGRIDEARAVLETIRPLERAHAEVADVEHLAKEEHVISEKSMGLREILSSKWLVRILLVGIGLGVAQQLTGINSIMYYGQVVLIEAGFSENAALIANVAPGVIAVVGAFIALWMMDRINRRTTLITGYSLTTISHVLIGIASVAFPVGDPLRPYVILTLVVVFVGSMQTFLNVATWVMLSELFPLAMRGFAIGISVFFLWIANAFLGLFFPTIMEAVGLTGTFFMFAGIGVVALIFIYTQVPETRGRTLEEIDADVTSGVIFNKDIRKGKVH

SEQ ID NO: 4 - DNA, 1476 bp, Artificial Sequence
  Wild-type sugar porter family MFS transporter, iolT1 coding gene
atggctagtaccttcattcaggccgacagccctgaaaaaagtaagaagctgcccccactcacagaaggtccgtatagaaaacggctattctacgttgcactagttgcgacgttcggtggactgctcttcggatacgacaccggcgtaatcaacggtgcactcaacccaatgacacgtgagctcgggctaaccgcgttcactgagggtgttgtaacttcttctctgctgtttggtgcagcagctggtgcgatgtttttcggtcgtatttccgacaactggggtcgtcggaaaacaatcatctcacttgcagtagctttctttatcggcaccatgatctgcgtgtttgctccatcttttgcagtaatggttgtcggacgtgtgcttcttggactcgcagttggtggcgcttccactgttgtccctgtctacctggctgaacttgctccttttgaaatccgtggctcactggctggccgtaatgagttgatgattgttgttggtcagctcgcagcttttgtcatcaatgcgattattggaaatgtttttggacaccacgatggtgtgtggcgctacatgctggcaattgccgcaatcccagcaattgccctcttctttggaatgctccgagttccagaatccccacgctggcttgttgagcgaggacgcattgatgaggctcgcgcagttcttgaaaccattcgccctcttgaacgtgcccatgcagaagttgctgatgttgaacacctagcaaaagaagaacatgtcatttccgagaagtccatgggcttaagggaaattttgtccagcaagtggcttgtgcgcatcctcctggtaggtatcggattgggtgtcgcacagcagctgaccggcattaactccatcatgtattacggccaggttgttctcattgaggctggtttctccgaaaatgcagctctgatcgccaacgtggcacctggagttatcgcagttgtcggtgcattcatcgcactgtggatgatggatcgcatcaaccgccgtaccaccctcattaccggctactctctcaccaccattagccacgtgttgatcggcatcgcatccgtagcattcccagttggcgatccacttcgcccatacgttatcttgactctagttgtggtcttcgtaggatccatgcagaccttcctcaacgtagccacctgggtcatgctctccgagctcttcccgctggcaatgcgcggtttcgcaatcggtatctcagtgttcttcctttggatcgcaaacgcgttcctcggattgttcttcccaaccatcatggaagcagtaggactaaccggaaccttcttcatgttcgccggaatcggtgtggttgccttgatcttcatctacacccaggttccagaaacccgtggacgcaccttggaggagatcgatgcggatgttacttccggagtcatcttcaacaaggatatccggaagggaaaggtgcactaa

SEQ ID NO: 5 - DNA, 40 bp, Artificial Sequence
  iolT1_1F
tgaattcgagctcggtaccctgtctacctggctgaacttg

SEQ ID NO: 6 - DNA, 33 bp, Artificial Sequence
  iolT1_2R
tccaggtgccacgttgacgatcagagctgcatt

SEQ ID NO: 7 - DNA, 33 bp, Artificial Sequence
  iolT1_3F
aatgcagctctgatcgtcaacgtggcacctgga

SEQ ID NO: 8 - DNA, 40 bp, Artificial Sequence
  iolT1_4R
gtcgactctagaggatccccatatccttgttgaagatgac

SEQ ID NO: 9 - DNA, 20 bp, Artificial Sequence
  iolT1_5F
tgtctacctggctgaacttg

SEQ ID NO: 10 - DNA, 20 bp, Artificial Sequence
  iolT1_6R
atatccttgttgaagatgac